European Patent Specification EP 4 092 114 B1, published August 28, 2024. Title: Novel 2-isopropylmalate synthase variant and a method for producing L-valine using the same. Applicant: CJ CheilJedang Corporation. The sequence listing filed with the application follows.

SEQUENCE LISTING (10 sequences)

SEQ ID NO: 1 - protein, 616 aa, Artificial Sequence
  2-isopropylmalate synthase variant
MSPNDAFISAPAKIETPVGPRNEGQPAWNKQRGSSMPVNRYMPFEVEVEDISLPDRTWPDKKITVAPQWCAVDLRDGNQALIDPMSLERKRRMFELLVQMGFKEIEVGFPSASQTDFDFVREIIEKDMIPDDVTIQVLVQAREHLIRRTFEACEGAKNVIVHFYNSTSILQRNVVFRMDKVQVKKLATDAAELIKTVAQDYPDTNWRWQYSPESFTGTEVEYAKEVVDAVVEVMDPTPENPMIINLPSTVEMITPNVYADSIEWMHRNLNRRDSIILSLHPHNDRGTGVGAAELGYMAGADRIEGCLFGNGERTGNVCLVTLALNMLTQGVDPQLDFTDIRQIRSTVEYCNQLRVPERHPYGGDLVFTAFSGSHQDAVNKGLDAMAAKVQPGASSTEVSWEQLRDTEWEVPYLPIDPKDVGRDYEAVIRVNSQSGKGGVAYIMKTDHGLQIPRSMQVEFSTVVQNVTDAEGGEVNSKAMWDIFATEYLERTAPVEQIALRVENAQTENEDASITAELIHNGKDVTVDGHGNGPLAAYANALEKLGIDVEIQEYNQHARTSGDDAEAAAYVLAEVNGRKVWGVGIAGSITYASLKAVTSAVNRALDVNHEAVLAGGV

SEQ ID NO: 2 - DNA, 1851 bp, Artificial Sequence
  2-isopropylmalate synthase variant coding gene
atgtctcctaacgatgcattcatctccgcacctgccaagatcgaaaccccagttgggcctcgcaatgaaggccagccagcatggaataagcagcgtggctcctcaatgccagttaaccgctacatgcctttcgaggttgaggtagaagatatttctctgccggaccgcacttggccagataaaaaaatcaccgttgcacctcagtggtgtgctgttgacctgcgtgacggcaaccaggctctgattgatccgatgtctcttgagcgtaagcgccgcatgtttgagctgctggttcagatgggattcaaggaaatcgaggtcggtttcccttcagcttcccagactgattttgatttcgttcgtgagatcatcgaaaaggacatgatccctgacgatgtcaccattcaggttctggttcaggctcgtgagcacctgattcgccgtacttttgaagcttgcgaaggcgcaaaaaacgttatcgtgcacttctacaactcaacctccatcctgcagcgcaacgtggtgttccgcatggacaaggtgcaggtgaagaagctggctaccgatgccgctgaactgatcaagaccgtcgctcaggattacccagacaccaactggcgctggcagtactcccctgagtccttcaccggcactgaggttgagtacgccaaggaagttgtggacgcagttgttgaggtcatggatccaactcctgagaacccaatgatcatcaacctgccttccaccgttgagatgatcacccctaacgtttacgcagactccattgaatggatgcaccgcaatctaaaccgtcgtgattccattatcctgtccctgcacccgcacaatgaccgtggcaccggcgttggcgcagctgagctgggctacatggctggcgctgaccgcatcgaaggctgcctgttcggcaacggcgagcgcaccggcaacgtctgcctggtcaccctggcactgaacatgctgacccagggcgttgaccctcagctggacttcaccgatatacgccagatccgcagcaccgttgaatactgcaaccagctgcgcgttcctgagcgccacccatacggcggcgacctggtcttcaccgctttctccggttcccaccaggacgctgtgaacaagggtctggacgccatggctgccaaggttcagccaggtgctagctccactgaagtttcttgggagcagctgcgcgacaccgaatgggaggttccttacctgcctatcgatccaaaggatgtcggtcgcgactacgaggctgttatccgcgtgaactcccagtccggcaagggcggcgttgcttacatcatgaagaccgatcacggtctgcagatccctcgctccatgcaggttgagttctccaccgttgtccagaacgtcaccgacgctgagggcggcgaggtcaactccaaggcaatgtgggatatcttcgccaccgagtacctggagcgcaccgcaccagttgagcagatcgcgctgcgcgtcgagaacgctcagaccgaaaacgaggatgcatccatcaccgccgagctcatccacaacggcaaggacgtcaccgtcgatggccacggcaacggcccactggctgcttacgccaacgcgctggagaagctgggcatcgacgttgagatccaggaatacaaccagcacgcccgcacctcgggcgacgatgcagaagcagccgcctacgtgctggctgaggtcaacggccgcaaggtctggggcgtcggcatcgctggctccatcacctacgcttcgctgaaggcagtgacctccgccgtaaaccgcgcgctggacgtcaaccacgaggcagtcctggctggcggcgtttaa

SEQ ID NO: 3 - protein, 616 aa, Artificial Sequence
  Wild-type 2-isopropylmalate synthase
MSPNDAFISAPAKIETPVGPRNEGQPAWNKQRGSSMPVNRYMPFEVEVEDISLPDRTWPDKKITVAPQWCAVDLRDGNQALIDPMSPERKRRMFELLVQMGFKEIEVGFPSASQTDFDFVREIIEKDMIPDDVTIQVLVQAREHLIRRTFEACEGAKNVIVHFYNSTSILQRNVVFRMDKVQVKKLATDAAELIKTVAQDYPDTNWRWQYSPESFTGTEVEYAKEVVDAVVEVMDPTPENPMIINLPSTVEMITPNVYADSIEWMHRNLNRRDSIILSLHPHNDRGTGVGAAELGYMAGADRIEGCLFGNGERTGNVCLVTLALNMLTQGVDPQLDFTDIRQIRSTVEYCNQLRVPERHPYGGDLVFTAFSGSHQDAVNKGLDAMAAKVQPGASSTEVSWEQLRDTEWEVPYLPIDPKDVGRDYEAVIRVNSQSGKGGVAYIMKTDHGLQIPRSMQVEFSTVVQNVTDAEGGEVNSKAMWDIFATEYLERTAPVEQIALRVENAQTENEDASITAELIHNGKDVTVDGHGNGPLAAYANALEKLGIDVEIQEYNQHARTSGDDAEAAAYVLAEVNGRKVWGVGIAGSITYASLKAVTSAVNRALDVNHEAVLAGGV

SEQ ID NO: 4 - DNA, 1851 bp, Artificial Sequence
  Wild-type 2-isopropylmalate synthase coding gene
atgtctcctaacgatgcattcatctccgcacctgccaagatcgaaaccccagttgggcctcgcaatgaaggccagccagcatggaataagcagcgtggctcctcaatgccagttaaccgctacatgcctttcgaggttgaggtagaagatatttctctgccggaccgcacttggccagataaaaaaatcaccgttgcacctcagtggtgtgctgttgacctgcgtgacggcaaccaggctctgattgatccgatgtctcctgagcgtaagcgccgcatgtttgagctgctggttcagatgggattcaaggaaatcgaggtcggtttcccttcagcttcccagactgattttgatttcgttcgtgagatcatcgaaaaggacatgatccctgacgatgtcaccattcaggttctggttcaggctcgtgagcacctgattcgccgtacttttgaagcttgcgaaggcgcaaaaaacgttatcgtgcacttctacaactcaacctccatcctgcagcgcaacgtggtgttccgcatggacaaggtgcaggtgaagaagctggctaccgatgccgctgaactgatcaagaccgtcgctcaggattacccagacaccaactggcgctggcagtactcccctgagtccttcaccggcactgaggttgagtacgccaaggaagttgtggacgcagttgttgaggtcatggatccaactcctgagaacccaatgatcatcaacctgccttccaccgttgagatgatcacccctaacgtttacgcagactccattgaatggatgcaccgcaatctaaaccgtcgtgattccattatcctgtccctgcacccgcacaatgaccgtggcaccggcgttggcgcagctgagctgggctacatggctggcgctgaccgcatcgaaggctgcctgttcggcaacggcgagcgcaccggcaacgtctgcctggtcaccctggcactgaacatgctgacccagggcgttgaccctcagctggacttcaccgatatacgccagatccgcagcaccgttgaatactgcaaccagctgcgcgttcctgagcgccacccatacggcggcgacctggtcttcaccgctttctccggttcccaccaggacgctgtgaacaagggtctggacgccatggctgccaaggttcagccaggtgctagctccactgaagtttcttgggagcagctgcgcgacaccgaatgggaggttccttacctgcctatcgatccaaaggatgtcggtcgcgactacgaggctgttatccgcgtgaactcccagtccggcaagggcggcgttgcttacatcatgaagaccgatcacggtctgcagatccctcgctccatgcaggttgagttctccaccgttgtccagaacgtcaccgacgctgagggcggcgaggtcaactccaaggcaatgtgggatatcttcgccaccgagtacctggagcgcaccgcaccagttgagcagatcgcgctgcgcgtcgagaacgctcagaccgaaaacgaggatgcatccatcaccgccgagctcatccacaacggcaaggacgtcaccgtcgatggccacggcaacggcccactggctgcttacgccaacgcgctggagaagctgggcatcgacgttgagatccaggaatacaaccagcacgcccgcacctcgggcgacgatgcagaagcagccgcctacgtgctggctgaggtcaacggccgcaaggtctggggcgtcggcatcgctggctccatcacctacgcttcgctgaaggcagtgacctccgccgtaaaccgcgcgctggacgtcaaccacgaggcagtcctggctggcggcgtttaa

SEQ ID NO: 5 - DNA, 40 bp, Artificial Sequence
  leuA_1F
tgaattcgagctcggtaccctgacagcactggaactgggc

SEQ ID NO: 6 - DNA, 33 bp, Artificial Sequence
  leuA_2R
gcggcgcttacgctcaagagacatcggatcaat

SEQ ID NO: 7 - DNA, 33 bp, Artificial Sequence
  leuA_3F
attgatccgatgtctcttgagcgtaagcgccgc

SEQ ID NO: 8 - DNA, 40 bp, Artificial Sequence
  leuA_4R
gtcgactctagaggatccccattcaatggagtctgcgtaa

SEQ ID NO: 9 - DNA, 20 bp, Artificial Sequence
  leuA_5F
tgacagcactggaactgggc

SEQ ID NO: 10 - DNA, 20 bp, Artificial Sequence
  leuA_6R
attcaatggagtctgcgtaa